European Patent Application EP 4 116 434 A1, published January 11, 2023. Title: IN VITRO METHOD FOR QUANTIFYING THE CELLULAR CONTENT OF SPECIFIC RNAs. Applicant: Universidad Autónoma de Madrid. The sequence listing filed with the application follows.

SEQUENCE LISTING (8 sequences)

SEQ ID NO: 1 - DNA, 29 bp, Artificial sequence
  Artificial sequence
gaactcgagtttgcgtgtcatccttgcgc

SEQ ID NO: 2 - DNA, 19 bp, Artificial sequence
  Artificial sequence
gaatcctgcgcaccgagat

SEQ ID NO: 3 - DNA, 22 bp, Artificial sequence
  Artificial sequence
ctgcacttgaaccctgcaatac

SEQ ID NO: 4 - DNA, 26 bp, Artificial sequence
  Artificial sequence
tctaaccctaactgagaagggcgtag

SEQ ID NO: 5 - DNA, 26 bp, Artificial sequence
  Artificial sequence
gtttgctctagaatgaacggtggaag

SEQ ID NO: 6 - DNA, 16 bp, Artificial sequence
  Artificial sequence
cacgtctatacaccac

SEQ ID NO: 7 - DNA, 15 bp, Artificial sequence
  Artificial sequence
taaccctaaccctaa

SEQ ID NO: 8 - DNA, 16 bp, Artificial sequence
  Artificial sequence
ctctagaatgaacggt